European Patent Application EP 4 717 771 A1, published April 1, 2026. Title: Reducing expression of proteinase 3 autoantigen in ANCA-associated vasculitis. Applicant: Charité - Universitätsmedizin Berlin Körperschaft des öffentlichen Rechts. The sequence listing filed with the application follows.

SEQUENCE LISTING (78 sequences)

SEQ ID NO: 1 - RNA, 20 nt, synthetic construct
  source 1..20: mol_type = other RNA
gcggccgtcagcacgaagct

SEQ ID NO: 2 - RNA, 20 nt, synthetic construct
  source 1..20: mol_type = other RNA
tgacggccgcgcactgcctg

SEQ ID NO: 3 - RNA, 20 nt, synthetic construct
  source 1..20: mol_type = other RNA
cggccgctcacatgtcccgc

SEQ ID NO: 4 - DNA, 23 bp, synthetic construct
  source 1..23: mol_type = other DNA
  misc_feature 1..3: note = Protospacer adjacent motif
  misc_feature 7: note = inserted base
cccagctttcgtgctgacggccg

SEQ ID NO: 5 - DNA, 23 bp, synthetic construct
  source 1..23: mol_type = other DNA
  misc_feature 18..20: note = mutated bases, n can be C, G, T or A
  misc_feature 21..23: note = Protospacer adjacent motif
tgacggccgcgcactgcnnngca

SEQ ID NO: 6 - skipped

SEQ ID NO: 7 - DNA, 771 bp, Homo sapiens
  source 1..771: mol_type = genomic DNA
atggctcaccggccccccagccctgccctggcgtccgtgctgctggccttgctgctgagcggtgctgcccgagctgcggagatcgtgggcgggcacgaggcgcagccacactcccggccctacatggcctccctgcagatgcgggggaacccgggcagccacttctgcggaggcaccttgatccaccccagcttcgtgctgacggccgcgcactgcctgcgggacataccccagcgcctggtgaacgtggtgctcggagcccacaacgtgcggacgcaggagcccacccagcagcacttctcggtggctcaggtgtttctgaacaactacgacgcggagaacaaactgaacgacgttctcctcatccagctgagcagcccagccaacctcagtgcctccgtcgccacagtccagctgccacagcaggaccagccagtgccccacggcacccagtgcctggccatgggctggggccgcgtgggtgcccacgaccccccagcccaggtcctgcaggagctcaatgtcaccgtggtcaccttcttctgccggccacataacatttgcactttcgtccctcgccgcaaggccggcatctgcttcggagactcaggtggccccctgatctgtgatggcatcatccaaggaatagactccttcgtgatctggggatgtgccacccgccttttccctgacttcttcacgcgggtagccctctacgtggactggatccgttccacgctgcgccgtgtggaggccaagggccgcccctga

SEQ ID NO: 8 - DNA, 20 bp, Homo sapiens
  source 1..20: mol_type = genomic DNA
gctgcccgagctgcggagat

SEQ ID NO: 9 - DNA, 20 bp, Homo sapiens
  source 1..20: mol_type = genomic DNA
tgcccgagctgcggagatcg

SEQ ID NO: 10 - DNA, 20 bp, Homo sapiens
  source 1..20: mol_type = genomic DNA
acgaggcgcagccacactcc

SEQ ID NO: 11 - DNA, 20 bp, Homo sapiens
  source 1..20: mol_type = genomic DNA
cctgcagatgcgggggaacc

SEQ ID NO: 12 - DNA, 20 bp, Homo sapiens
  source 1..20: mol_type = genomic DNA
agaccccagcgcctggtgaa

SEQ ID NO: 13 - DNA, 20 bp, Homo sapiens
  source 1..20: mol_type = genomic DNA
accccagcgcctggtgaacg

SEQ ID NO: 14 - DNA, 20 bp, Homo sapiens
  source 1..20: mol_type = genomic DNA
gcggacgcaggagcccaccc

SEQ ID NO: 15 - DNA, 20 bp, Homo sapiens
  source 1..20: mol_type = genomic DNA
gcccacccagcagcacttct

SEQ ID NO: 16 - DNA, 20 bp, Homo sapiens
  source 1..20: mol_type = genomic DNA
cccacccagcagcacttctc

SEQ ID NO: 17 - DNA, 20 bp, Homo sapiens
  source 1..20: mol_type = genomic DNA
cacccagcagcacttctcgg

SEQ ID NO: 18 - DNA, 20 bp, Homo sapiens
  source 1..20: mol_type = genomic DNA
cctcatccaggtgggcgggc

SEQ ID NO: 19 - DNA, 20 bp, Homo sapiens
  source 1..20: mol_type = genomic DNA
cacagtccagctgccacagc

SEQ ID NO: 20 - DNA, 20 bp, Homo sapiens
  source 1..20: mol_type = genomic DNA
ctgccacagcaggaccagcc

SEQ ID NO: 21 - DNA, 20 bp, Homo sapiens
  source 1..20: mol_type = genomic DNA
caggaccagccagtgcccca

SEQ ID NO: 22 - DNA, 20 bp, Homo sapiens
  source 1..20: mol_type = genomic DNA
cggcacccagtgcctggcca

SEQ ID NO: 23 - DNA, 20 bp, Homo sapiens
  source 1..20: mol_type = genomic DNA
gcggccccagcccatggcca

SEQ ID NO: 24 - DNA, 20 bp, Homo sapiens
  source 1..20: mol_type = genomic DNA
cgcggccccagcccatggcc

SEQ ID NO: 25 - DNA, 20 bp, Homo sapiens
  source 1..20: mol_type = genomic DNA
cccccagcccaggtcctgca

SEQ ID NO: 26 - DNA, 20 bp, Homo sapiens
  source 1..20: mol_type = genomic DNA
caggtcctgcaggagctcaa

SEQ ID NO: 27 - DNA, 20 bp, Homo sapiens
  source 1..20: mol_type = genomic DNA
atccaaggaatagactcctt

SEQ ID NO: 28 - DNA, 20 bp, Homo sapiens
  source 1..20: mol_type = genomic DNA
acatccccagatcacgaagg

SEQ ID NO: 29 - DNA, 20 bp, Homo sapiens
  source 1..20: mol_type = genomic DNA
ggcacatccccagatcacga

SEQ ID NO: 30 - DNA, 20 bp, Homo sapiens
  source 1..20: mol_type = genomic DNA
cggatccagtccacgtagag

SEQ ID NO: 31 - DNA, 20 bp, Homo sapiens
  source 1..20: mol_type = genomic DNA
acggatccagtccacgtaga

SEQ ID NO: 32 - DNA, 23 bp, Homo sapiens
  source 1..23: mol_type = genomic DNA
cctgcagcctgggggctccctga

SEQ ID NO: 33 - DNA, 23 bp, Homo sapiens
  source 1..23: mol_type = genomic DNA
tgaacaactacgacgcggagaac

SEQ ID NO: 34 - DNA, 23 bp, Homo sapiens
  source 1..23: mol_type = genomic DNA
ttctccgcgtcgtagttgttcag

SEQ ID NO: 35 - DNA, 23 bp, Homo sapiens
  source 1..23: mol_type = genomic DNA
cactttcgtccctcgccgcaagg

SEQ ID NO: 36 - DNA, 23 bp, Homo sapiens
  source 1..23: mol_type = genomic DNA
gtccctcgccgcaaggccggcat

SEQ ID NO: 37 - DNA, 23 bp, Homo sapiens
  source 1..23: mol_type = genomic DNA
ccctgacttcttcacgcgggtag

SEQ ID NO: 38 - DNA, 23 bp, Homo sapiens
  source 1..23: mol_type = genomic DNA
cctgacttcttcacgcgggtagc

SEQ ID NO: 39 - DNA, 23 bp, Homo sapiens
  source 1..23: mol_type = genomic DNA
gagccaggctcggggtcccggcc

SEQ ID NO: 40 - DNA, 23 bp, Homo sapiens
  source 1..23: mol_type = genomic DNA
gacagaagcagctcttccccgaa

SEQ ID NO: 41 - DNA, 23 bp, Homo sapiens
  source 1..23: mol_type = genomic DNA
ttgaggtcacggtggggtgaggt

SEQ ID NO: 42 - DNA, 23 bp, Homo sapiens
  source 1..23: mol_type = genomic DNA
aacgtttattgaggtcacggtgg

SEQ ID NO: 43 - skipped

SEQ ID NO: 44 - DNA, 20 bp, Homo sapiens
  source 1..20: mol_type = genomic DNA
ggggtctgcgggggtggggt

SEQ ID NO: 45 - DNA, 20 bp, Homo sapiens
  source 1..20: mol_type = genomic DNA
tctccctggaggacagggac

SEQ ID NO: 46 - DNA, 20 bp, Homo sapiens
  source 1..20: mol_type = genomic DNA
gcccacctggatgaggagaa

SEQ ID NO: 47 - DNA, 20 bp, Homo sapiens
  source 1..20: mol_type = genomic DNA
tggggtctgcgggggtgggg

SEQ ID NO: 48 - DNA, 20 bp, Homo sapiens
  source 1..20: mol_type = genomic DNA
gtctccctggaggacaggga

SEQ ID NO: 49 - DNA, 20 bp, Homo sapiens
  source 1..20: mol_type = genomic DNA
ctcacatgtcccgcaggcag

SEQ ID NO: 50 - DNA, 20 bp, Homo sapiens
  source 1..20: mol_type = genomic DNA
cgctcacatgtcccgcaggc

SEQ ID NO: 51 - DNA, 20 bp, Homo sapiens
  source 1..20: mol_type = genomic DNA
cactcaccgctcagcagcaa

SEQ ID NO: 52 - DNA, 20 bp, Homo sapiens
  source 1..20: mol_type = genomic DNA
ctcagctggggcagaaggca

SEQ ID NO: 53 - DNA, 20 bp, Homo sapiens
  source 1..20: mol_type = genomic DNA
gctggggtctgcgggggtgg

SEQ ID NO: 54 - DNA, 20 bp, Homo sapiens
  source 1..20: mol_type = genomic DNA
tcactcaccgctcagcagca

SEQ ID NO: 55 - DNA, 20 bp, Homo sapiens
  source 1..20: mol_type = genomic DNA
cacctgcagggggggagtcc

SEQ ID NO: 56 - DNA, 20 bp, Homo sapiens
  source 1..20: mol_type = genomic DNA
cgctggggtctgcgggggtg

SEQ ID NO: 57 - DNA, 20 bp, Homo sapiens
  source 1..20: mol_type = genomic DNA
tgagtctccctggaggacag

SEQ ID NO: 58 - DNA, 20 bp, Homo sapiens
  source 1..20: mol_type = genomic DNA
ttacttacgaagcagatgcc

SEQ ID NO: 59 - DNA, 20 bp, Homo sapiens
  source 1..20: mol_type = genomic DNA
ggcagcacctgcaggggggg

SEQ ID NO: 60 - DNA, 20 bp, Homo sapiens
  source 1..20: mol_type = genomic DNA
gcccgcccacctggatgagg

SEQ ID NO: 61 - DNA, 20 bp, Homo sapiens
  source 1..20: mol_type = genomic DNA
ggccgctcacatgtcccgca

SEQ ID NO: 62 - DNA, 20 bp, Homo sapiens
  source 1..20: mol_type = genomic DNA
gttacttacgaagcagatgc

SEQ ID NO: 63 - DNA, 20 bp, Homo sapiens
  source 1..20: mol_type = genomic DNA
gctcagctggggcagaaggc

SEQ ID NO: 64 - DNA, 20 bp, Homo sapiens
  source 1..20: mol_type = genomic DNA
cggccgctcacatgtcccgc

SEQ ID NO: 65 - DNA, 20 bp, Homo sapiens
  source 1..20: mol_type = genomic DNA
cagctggggcagaaggcagg

SEQ ID NO: 66 - DNA, 20 bp, Homo sapiens
  source 1..20: mol_type = genomic DNA
gctgctcagctggggcagaa

SEQ ID NO: 67 - DNA, 20 bp, Homo sapiens
  source 1..20: mol_type = genomic DNA
ccccctgcaggtgctgcccg

SEQ ID NO: 68 - DNA, 20 bp, Homo sapiens
  source 1..20: mol_type = genomic DNA
cctgcaggtgctgcccgagc

SEQ ID NO: 69 - DNA, 20 bp, Homo sapiens
  source 1..20: mol_type = genomic DNA
tgcaggtgctgcccgagctg

SEQ ID NO: 70 - DNA, 20 bp, Homo sapiens
  source 1..20: mol_type = genomic DNA
cccccgcagaccccagcgcc

SEQ ID NO: 71 - DNA, 20 bp, Homo sapiens
  source 1..20: mol_type = genomic DNA
ccccgcagaccccagcgcct

SEQ ID NO: 72 - DNA, 20 bp, Homo sapiens
  source 1..20: mol_type = genomic DNA
ccgcagaccccagcgcctgg

SEQ ID NO: 73 - DNA, 20 bp, Homo sapiens
  source 1..20: mol_type = genomic DNA
ctgccccagctgagcagccc

SEQ ID NO: 74 - DNA, 20 bp, Homo sapiens
  source 1..20: mol_type = genomic DNA
ctgtcctccagggagactca

SEQ ID NO: 75 - DNA, 20 bp, Homo sapiens
  source 1..20: mol_type = genomic DNA
gtcctccagggagactcagg

SEQ ID NO: 76 - DNA, 20 bp, Homo sapiens
  source 1..20: mol_type = genomic DNA
tcctccagggagactcaggt

SEQ ID NO: 77 - DNA, 20 bp, synthetic construct
  source 1..20: mol_type = other DNA
gagtccttcccaccagccag

SEQ ID NO: 78 - DNA, 20 bp, synthetic construct
  source 1..20: mol_type = other DNA
ctccgagcaccacgttcacc